European Patent Application EP 4 744 730 A2, published May 20, 2026. Title: TARGETED IL-12 TREATMENTS AND METHODS TO STIMULATE HANK AND NK92MI CELLS. Applicant: NantBio, Inc. The sequence listing filed with the application follows.

SEQUENCE LISTING (3 sequences)

SEQ ID NO: 1 - protein, 994 aa, synthetic construct
  source 1..994: note = Chimeric Sequence for leader peptide/mouse scIL-12/hu51-4 heavy chain
MCHQQLVISWFSLVFLASPLMWELEKDVYVVEVDWTPDAPGETVNLTCDTPEEDDITWTSDQRHGVIGSGKTLTITVKEFLDAGQYTCHKGGETLSHSHLLLHKKENGIWSTEILKNFKNKTFLKCEAPNYSGRFTCSWLVQRNMDLKFNIKSSSSSPDSRAVTCGMASLSAEKVTLDQRDYEKYSVSCQEDVTCPTAEETLPIELALEARQQNKYENYSTSFFIRDIIKPDPPKNLQMKPLKNSQVEVSWEYPDSWSTPHSYFSLKFFVRIQRKKEKMKETEEGCNQKGAFLVEKTSTEVQCKGGNVCVQAQDRYYNSSCSKWACVPCRVRSGGGGSGGGGSGGGGSRVIPVSGPARCLSQSRNLLKTTDDMVKTAREKLKHYSCTAEDIDHKDITRDQTSTLKTCLPLELHKNESCLATRETSSTTRGSCLPPQKTSLMMTLCLGSIYEDLKMYQTEFQAINAALQNHNHQQIILDKGMLVAIDELMQSLNHNGETLRQKPPVGEADPYRVKMKLCILLHAFSTRVVTINRVMGYLSSALEQVQLVQSGAEVKKPGASVKVSCKASGYTFTRYWMHWVRQAPGQGLEWIGAIYPGNSDTSYNQKFKGKATITADTSTNTAYMELSSLRSEDTAVYYCARGEEIGSRRWFAYWGQGTLVTVSSASTKGPSVFPLAPSSKSTSGGTAALGCLVKDYFPEPVTVSWNSGALTSGVHTFPAVLQSSGLYSLSSVVTVPSSSLGTQTYICNVNHKPSNTKVDKKVEPKSCDKTHTCPPCPAPELLGGPSVFLFPPKPKDTLMISRTPEVTCVVVDVSHEDPEVKFNWYVDGVEVHNAKTKPREEQYNSTYRVVSVLTVLHQDWLNGKEYKCKVSNKALPAPIEKTISKAKGQPREPQVYTLPPSRDELTKNQVSLTCLVKGFYPSDIAVEWESNGQPENNYKTTPPVLDSDGSFFLYSKLTVDKSRWQQGNVFSCSVMHEALHNHYTQKSLSLSPGK

SEQ ID NO: 2 - protein, 991 aa, synthetic construct
  source 1..991: note = Chimeric Sequence for leader peptide/human scIL-12/hu51-4 heavy chain
MCHQQLVISWFSLVFLASPLIWELKKDVYVVELDWYPDAPGEMVVLTCDTPEEDGITWTLDQSSEVLGSGKTLTIQVKEFGDAGQYTCHKGGEVLSHSLLLLHKKEDGIWSTDILKDQKEPKNKTFLRCEAKNYSGRFTCWWLTTISTDLTFSVKSSRGSSDPQGVTCGAATLSAERVRGDNKEYEYSVECQEDSACPAAEESLPIEVMVDAVHKLKYENYTSSFFIRDIIKPDPPKNLQLKPLKNSRQVEVSWEYPDTWSTPHSYFSLTFCVQVQGKSKREKKDRVFTDKTSATVICRKNASISVRAQDRYYSSSWSEWASVPCSGGGGSGGGGSGGGGSRNLPVATPDPGMFPCLHHSQNLLRAVSNMLQKARQTLEFYPCTSEEIDHEDITKDKTSTVEACLPLELTKNESCLNSRETSFITNGSCLASRKTSFMMALCLSSIYEDLKMYQVEFKTMNAKLLMDPKRQIFLDQNMLAVIDELMQALNFNSETVPQKSSLEEPDFYKTKIKLCILLHAFRIRAVTIDRVMSYLNASLEQVQLVQSGAEVKKPGASVKVSCKASGYTFTRYWMHWVRQAPGQGLEWIGAIYPGNSDTSYNQKFKGKATITADTSTNTAYMELSSLRSEDTAVYYCARGEEIGSRRWFAYWGQGTLVTVSSASTKGPSVFPLAPSSKSTSGGTAALGCLVKDYFPEPVTVSWNSGALTSGVHTFPAVLQSSGLYSLSSVVTVPSSSLGTQTYICNVNHKPSNTKVDKKVEPKSCDKTHTCPPCPAPELLGGPSVFLFPPKPKDTLMISRTPEVTCVVVDVSHEDPEVKFNWYVDGVEVHNAKTKPREEQYNSTYRVVSVLTVLHQDWLNGKEYKCKVSNKALPAPIEKTISKAKGQPREPQVYTLPPSRDELTKNQVSLTCLVKGFYPSDIAVEWESNGQPENNYKTTPPVLDSDGSFFLYSKLTVDKSRWQQGNVFSCSVMHEALHNHYTQKSLSLSPGK

SEQ ID NO: 3 - protein, 236 aa, synthetic construct
  source 1..236: note = Chimeric Sequence for leader peptide/hu51-4 light chain
MDFQVQIFSFLLISASVAMSRGEIVLTQSPATLSLSPGERATLSCRARQSISNYLHWYQQKPGQAPRLLIYYASQSISGIPDRFSGSGSGTDFTLTISRLEPEDFAVYYCQQSNSWPLTFGQGTKVEIKRTVAAPSVFIFPPSDEQLKSGTASVVCLLNNFYPREAKVQWKVDNALQSGNSQESVTEQDSKDSTYSLSSTLTLSKADYEKHKVYACEVTHQGLSSPVTKSFNRGEC